European Patent Specification EP 4 429 690 B1, published May 13, 2026. Title: A chimeric endolysin polypeptide. Applicant: Micreos Pharmaceuticals AG. The sequence listing filed with the application follows.

SEQUENCE LISTING (161 sequences)

SEQ ID NO: 1 - protein, 417 aa, synthetic construct
MKTLKQAESYIKSKVNTGTDFDGLYGYQCMDLAVDYIYHVTDGKIRMWGNAKDAINNSFGGTATVYKNYPAFRPKYGDVVVWTTGNFATYGHIAIVTNPDPYGDLQYVTVLEQNWNGNGIYKTELATIRTHDYTGITHFIRPNFATESSVKKKDTKKKPKPSNRDGINKDKAATHEHSAQWLNNYKKGYGYGPYPLGINGGMHYGVDFFMNIGTPVKAISSGKIVEAGWSNYGGGNQIGLIENDGVHRQWYMHLSKYNVKVGDYVKAGQIIGWSGSTGYSTAPHLHFQRMVNSFSNSTAQDPMPFLKSAGYGKAGGTVTPTPNTGWKTNKYGTLYKSESASFTPNTDIITRTTGPFRSMPQSGVLKAGQTIHYDEVMKQDGHVWVGYTGNSGQRIYLPVRTWNKSTNTLGVLWGTIK

SEQ ID NO: 2 - protein, 403 aa, synthetic construct
MKTLKQAESYIKSKVNTGTDFDGLYGYQCMDLAVDYIYHVTDGKIRMWGNAKDAINNSFGGTATVYKNYPAFRPKYGDVVVWTTGNFATYGHIAIVTNPDPYGDLQYVTVLEQNWNGNGIYKTELATIRTHDYTGITHFIRPNFATESSNSTSSSNNNGAATHEHSAQWLNNYKKGYGYGPYPLGINGGMHYGVDFFMNIGTPVKAISSGKIVEAGWSNYGGGNQIGLIENDGVHRQWYMHLSKYNVKVGDYVKAGQIIGWSGSTGYSTAPHLHFQRMVNSFSNSTAQDPMPFLKSAGYGSNSTSSSNNNGWKTNKYGTLYKSESASFTPNTDIITRTTGPFRSMPQSGVLKAGQTIHYDEVMKQDGHVWVGYTGNSGQRIYLPVRTWNKSTNTLGVLWGTIK

SEQ ID NO: 3 - protein, 439 aa, synthetic construct
MKTLKQAESYIKSKVNTGTDFDGLYGYQCMDLAVDYIYHVTDGKIRMWGNAKDAINNSFGGTATVYKNYPAFRPKYGDVVVWTTGNFATYGHIAIVTNPDPYGDLQYVTVLEQNWNGNGIYKTELATIRTHDYTGITHFIRPNFATESSVKKKDTKKKPKPSNRDGINKDKAATHEHSAQWLNNYKKGYGYGPYPLGINGGMHYGVDFFMNIGTPVKAISSGKIVEAGWSNYGGGNQIGLIENDGVHRQWYMHLSKYNVKVGDYVKAGQIIGWSGSTGYSTAPHLHFQRMVNSFSNSTAQDPMPFLKSAGYGGKLEVSKAATIKQSDVKQEVKKQEAKQIVKATDWKQNKDGIWYKAEHASFTVTAPEGIITRYKGPWTGHPQAGVLQKGQTIKYDEVQKFDGHVWVSWETFEGETVYMPVRTWDAKTGKVGKLWGEIK

SEQ ID NO: 4 - protein, 148 aa, synthetic construct
MKTLKQAESYIKSKVNTGTDFDGLYGYQCMDLAVDYIYHVTDGKIRMWGNAKDAINNSFGGTATVYKNYPAFRPKYGDVVVWTTGNFATYGHIAIVTNPDPYGDLQYVTVLEQNWNGNGIYKTELATIRTHDYTGITHFIRPNFATES

SEQ ID NO: 5 - protein, 141 aa, synthetic construct
AATHEHSAQWLNNYKKGYGYGPYPLGINGGMHYGVDFFMNIGTPVKAISSGKIVEAGWSNYGGGNQIGLIENDGVHRQWYMHLSKYNVKVGDYVKAGQIIGWSGSTGYSTAPHLHFQRMVNSFSNSTAQDPMPFLKSAGYG

SEQ ID NO: 6 - protein, 92 aa, synthetic construct
WKTNKYGTLYKSESASFTPNTDIITRTTGPFRSMPQSGVLKAGQTIHYDEVMKQDGHVWVGYTGNSGQRIYLPVRTWNKSTNTLGVLWGTIK

SEQ ID NO: 7 - protein, 94 aa, synthetic construct
WKQNKDGIWYKAEHASFTVTAPEGIITRYKGPWTGHPQAGVLQKGQTIKYDEVQKFDGHVWVSWETFEGETVYMPVRTWDAKTGKVGKLWGEIK

SEQ ID NO: 8 - protein, 23 aa, synthetic construct
SVKKKDTKKKPKPSNRDGINKDK

SEQ ID NO: 9 - protein, 13 aa, synthetic construct
KAGGTVTPTPNTG

SEQ ID NO: 10 - protein, 11 aa, synthetic construct
SNSTSSSNNNG

SEQ ID NO: 11 - protein, 33 aa, synthetic construct
GKLEVSKAATIKQSDVKQEVKKQEAKQIVKATD

SEQ ID NO: 12 - protein, 23 aa, synthetic construct
SVKKKDTKKKPKPSNRDGINKDK

SEQ ID NO: 13 - protein, 22 aa, synthetic construct
VKKKDTKKKPKPSNRDGINKDK

SEQ ID NO: 14 - protein, 21 aa, synthetic construct
KKKDTKKKPKPSNRDGINKDK

SEQ ID NO: 15 - protein, 20 aa, unidentified
KKDTKKKPKPSNRDGINKDK

SEQ ID NO: 16 - protein, 19 aa, synthetic construct
KDTKKKPKPSNRDGINKDK

SEQ ID NO: 17 - protein, 18 aa, synthetic construct
DTKKKPKPSNRDGINKDK

SEQ ID NO: 18 - protein, 17 aa, synthetic construct
TKKKPKPSNRDGINKDK

SEQ ID NO: 19 - protein, 16 aa, synthetic construct
KKKPKPSNRDGINKDK

SEQ ID NO: 20 - protein, 15 aa, synthetic construct
KKPKPSNRDGINKDK

SEQ ID NO: 21 - protein, 14 aa, unidentified
KPKPSNRDGINKDK

SEQ ID NO: 22 - protein, 13 aa, synthetic construct
PKPSNRDGINKDK

SEQ ID NO: 23 - protein, 12 aa, synthetic construct
KPSNRDGINKDK

SEQ ID NO: 24 - protein, 11 aa, synthetic construct
PSNRDGINKDK

SEQ ID NO: 25 - protein, 10 aa, synthetic construct
SNRDGINKDK

SEQ ID NO: 26 - protein, 22 aa, synthetic construct
SVKKKDTKKKPKPSNRDGINKD

SEQ ID NO: 27 - protein, 21 aa, synthetic construct
VKKKDTKKKPKPSNRDGINKD

SEQ ID NO: 28 - protein, 20 aa, synthetic construct
KKKDTKKKPKPSNRDGINKD

SEQ ID NO: 29 - protein, 19 aa, synthetic construct
KKDTKKKPKPSNRDGINKD

SEQ ID NO: 30 - protein, 18 aa, synthetic construct
KDTKKKPKPSNRDGINKD

SEQ ID NO: 31 - protein, 17 aa, synthetic construct
DTKKKPKPSNRDGINKD

SEQ ID NO: 32 - protein, 16 aa, synthetic construct
TKKKPKPSNRDGINKD

SEQ ID NO: 33 - protein, 15 aa, synthetic construct
KKKPKPSNRDGINKD

SEQ ID NO: 34 - protein, 14 aa, synthetic construct
KKPKPSNRDGINKD

SEQ ID NO: 35 - protein, 13 aa, synthetic construct
KPKPSNRDGINKD

SEQ ID NO: 36 - protein, 12 aa, synthetic construct
PKPSNRDGINKD

SEQ ID NO: 37 - protein, 11 aa, synthetic construct
KPSNRDGINKD

SEQ ID NO: 38 - protein, 10 aa, synthetic construct
PSNRDGINKD

SEQ ID NO: 39 - protein, 21 aa, synthetic construct
SVKKKDTKKKPKPSNRDGINK

SEQ ID NO: 40 - protein, 20 aa, synthetic construct
VKKKDTKKKPKPSNRDGINK

SEQ ID NO: 41 - protein, 19 aa, synthetic construct
KKKDTKKKPKPSNRDGINK

SEQ ID NO: 42 - protein, 18 aa, synthetic construct
KKDTKKKPKPSNRDGINK

SEQ ID NO: 43 - protein, 17 aa, synthetic construct
KDTKKKPKPSNRDGINK

SEQ ID NO: 44 - protein, 16 aa, synthetic construct
DTKKKPKPSNRDGINK

SEQ ID NO: 45 - protein, 15 aa, synthetic construct
TKKKPKPSNRDGINK

SEQ ID NO: 46 - protein, 14 aa, synthetic construct
KKKPKPSNRDGINK

SEQ ID NO: 47 - protein, 13 aa, synthetic construct
KKPKPSNRDGINK

SEQ ID NO: 48 - protein, 12 aa, synthetic construct
KPKPSNRDGINK

SEQ ID NO: 49 - protein, 11 aa, synthetic construct
PKPSNRDGINK

SEQ ID NO: 50 - protein, 10 aa, unidentified
KPSNRDGINK

SEQ ID NO: 51 - protein, 20 aa, synthetic construct
SVKKKDTKKKPKPSNRDGIN

SEQ ID NO: 52 - protein, 19 aa, synthetic construct
VKKKDTKKKPKPSNRDGIN

SEQ ID NO: 53 - protein, 18 aa, synthetic construct
KKKDTKKKPKPSNRDGIN

SEQ ID NO: 54 - protein, 17 aa, synthetic construct
KKDTKKKPKPSNRDGIN

SEQ ID NO: 55 - protein, 16 aa, synthetic construct
KDTKKKPKPSNRDGIN

SEQ ID NO: 56 - protein, 15 aa, synthetic construct
DTKKKPKPSNRDGIN

SEQ ID NO: 57 - protein, 14 aa, synthetic construct
TKKKPKPSNRDGIN

SEQ ID NO: 58 - protein, 13 aa, synthetic construct
KKKPKPSNRDGIN

SEQ ID NO: 59 - protein, 12 aa, synthetic construct
KKPKPSNRDGIN

SEQ ID NO: 60 - protein, 11 aa, synthetic construct
KPKPSNRDGIN

SEQ ID NO: 61 - protein, 10 aa, synthetic construct
PKPSNRDGIN

SEQ ID NO: 62 - protein, 19 aa, synthetic construct
SVKKKDTKKKPKPSNRDGI

SEQ ID NO: 63 - protein, 18 aa, synthetic construct
VKKKDTKKKPKPSNRDGI

SEQ ID NO: 64 - protein, 17 aa, synthetic construct
KKKDTKKKPKPSNRDGI

SEQ ID NO: 65 - protein, 16 aa, synthetic construct
KKDTKKKPKPSNRDGI

SEQ ID NO: 66 - protein, 15 aa, synthetic construct
KDTKKKPKPSNRDGI

SEQ ID NO: 67 - protein, 14 aa, synthetic construct
DTKKKPKPSNRDGI

SEQ ID NO: 68 - protein, 13 aa, synthetic construct
TKKKPKPSNRDGI

SEQ ID NO: 69 - protein, 12 aa, synthetic construct
KKKPKPSNRDGI

SEQ ID NO: 70 - protein, 11 aa, synthetic construct
KKPKPSNRDGI

SEQ ID NO: 71 - protein, 10 aa, synthetic construct
KPKPSNRDGI

SEQ ID NO: 72 - protein, 18 aa, synthetic construct
SVKKKDTKKKPKPSNRDG

SEQ ID NO: 73 - protein, 17 aa, synthetic construct
VKKKDTKKKPKPSNRDG

SEQ ID NO: 74 - protein, 16 aa, synthetic construct
KKKDTKKKPKPSNRDG

SEQ ID NO: 75 - protein, 15 aa, synthetic construct
KKDTKKKPKPSNRDG

SEQ ID NO: 76 - protein, 14 aa, synthetic construct
KDTKKKPKPSNRDG

SEQ ID NO: 77 - protein, 13 aa, synthetic construct
DTKKKPKPSNRDG

SEQ ID NO: 78 - protein, 12 aa, synthetic construct
TKKKPKPSNRDG

SEQ ID NO: 79 - protein, 11 aa, synthetic construct
KKKPKPSNRDG

SEQ ID NO: 80 - protein, 10 aa, synthetic construct
KKPKPSNRDG

SEQ ID NO: 81 - protein, 17 aa, synthetic construct
SVKKKDTKKKPKPSNRD

SEQ ID NO: 82 - protein, 16 aa, synthetic construct
VKKKDTKKKPKPSNRD

SEQ ID NO: 83 - protein, 15 aa, synthetic construct
KKKDTKKKPKPSNRD

SEQ ID NO: 84 - protein, 14 aa, synthetic construct
KKDTKKKPKPSNRD

SEQ ID NO: 85 - protein, 13 aa, synthetic construct
KDTKKKPKPSNRD

SEQ ID NO: 86 - protein, 12 aa, synthetic construct
DTKKKPKPSNRD

SEQ ID NO: 87 - protein, 11 aa, synthetic construct
TKKKPKPSNRD

SEQ ID NO: 88 - protein, 10 aa, synthetic construct
KKKPKPSNRD

SEQ ID NO: 89 - protein, 16 aa, synthetic construct
SVKKKDTKKKPKPSNR

SEQ ID NO: 90 - protein, 15 aa, synthetic construct
VKKKDTKKKPKPSNR

SEQ ID NO: 91 - protein, 14 aa, synthetic construct
KKKDTKKKPKPSNR

SEQ ID NO: 92 - protein, 13 aa, synthetic construct
KKDTKKKPKPSNR

SEQ ID NO: 93 - protein, 12 aa, synthetic construct
KDTKKKPKPSNR

SEQ ID NO: 94 - protein, 11 aa, synthetic construct
DTKKKPKPSNR

SEQ ID NO: 95 - protein, 10 aa, synthetic construct
TKKKPKPSNR

SEQ ID NO: 96 - protein, 15 aa, synthetic construct
SVKKKDTKKKPKPSN

SEQ ID NO: 97 - protein, 14 aa, synthetic construct
VKKKDTKKKPKPSN

SEQ ID NO: 98 - protein, 13 aa, synthetic construct
KKKDTKKKPKPSN

SEQ ID NO: 99 - protein, 12 aa, synthetic construct
KKDTKKKPKPSN

SEQ ID NO: 100 - protein, 11 aa, synthetic construct
KDTKKKPKPSN

SEQ ID NO: 101 - protein, 10 aa, synthetic construct
DTKKKPKPSN

SEQ ID NO: 102 - protein, 14 aa, synthetic construct
SVKKKDTKKKPKPS

SEQ ID NO: 103 - protein, 13 aa, synthetic construct
VKKKDTKKKPKPS

SEQ ID NO: 104 - protein, 12 aa, synthetic construct
KKKDTKKKPKPS

SEQ ID NO: 105 - protein, 11 aa, synthetic construct
KKDTKKKPKPS

SEQ ID NO: 106 - protein, 10 aa, synthetic construct
KDTKKKPKPS

SEQ ID NO: 107 - protein, 13 aa, synthetic construct
SVKKKDTKKKPKP

SEQ ID NO: 108 - protein, 12 aa, synthetic construct
VKKKDTKKKPKP

SEQ ID NO: 109 - protein, 11 aa, synthetic construct
KKKDTKKKPKP

SEQ ID NO: 110 - protein, 10 aa, synthetic construct
KKDTKKKPKP

SEQ ID NO: 111 - protein, 12 aa, synthetic construct
SVKKKDTKKKPK

SEQ ID NO: 112 - protein, 11 aa, synthetic construct
VKKKDTKKKPK

SEQ ID NO: 113 - protein, 10 aa, synthetic construct
KKKDTKKKPK

SEQ ID NO: 114 - protein, 11 aa, synthetic construct
SVKKKDTKKKP

SEQ ID NO: 115 - protein, 10 aa, synthetic construct
VKKKDTKKKP

SEQ ID NO: 116 - protein, 10 aa, synthetic construct
SVKKKDTKKK

SEQ ID NO: 117 - protein, 13 aa, synthetic construct
KAGGTVTPTPNTG

SEQ ID NO: 118 - protein, 12 aa, synthetic construct
KAGGTVTPTPNT

SEQ ID NO: 119 - protein, 11 aa, synthetic construct
KAGGTVTPTPN

SEQ ID NO: 120 - protein, 10 aa, synthetic construct
KAGGTVTPTP

SEQ ID NO: 121 - protein, 9 aa, synthetic construct
KAGGTVTPT

SEQ ID NO: 122 - protein, 8 aa, synthetic construct
KAGGTVTP

SEQ ID NO: 123 - protein, 7 aa, synthetic construct
KAGGTVT

SEQ ID NO: 124 - protein, 6 aa, synthetic construct
KAGGTV

SEQ ID NO: 125 - protein, 5 aa, synthetic construct
KAGGT

SEQ ID NO: 126 - protein, 12 aa, synthetic construct
AGGTVTPTPNTG

SEQ ID NO: 127 - protein, 11 aa, synthetic construct
AGGTVTPTPNT

SEQ ID NO: 128 - protein, 10 aa, synthetic construct
AGGTVTPTPN

SEQ ID NO: 129 - protein, 9 aa, synthetic construct
AGGTVTPTP

SEQ ID NO: 130 - protein, 8 aa, synthetic construct
AGGTVTPT

SEQ ID NO: 131 - protein, 7 aa, synthetic construct
AGGTVTP

SEQ ID NO: 132 - protein, 6 aa, synthetic construct
AGGTVT

SEQ ID NO: 133 - protein, 5 aa, synthetic construct
AGGTV

SEQ ID NO: 134 - protein, 11 aa, synthetic construct
GGTVTPTPNTG

SEQ ID NO: 135 - protein, 10 aa, synthetic construct
GGTVTPTPNT

SEQ ID NO: 136 - protein, 9 aa, synthetic construct
GGTVTPTPN

SEQ ID NO: 137 - protein, 8 aa, synthetic construct
GGTVTPTP

SEQ ID NO: 138 - protein, 7 aa, synthetic construct
GGTVTPT

SEQ ID NO: 139 - protein, 6 aa, synthetic construct
GGTVTP

SEQ ID NO: 140 - protein, 5 aa, synthetic construct
GGTVT

SEQ ID NO: 141 - protein, 10 aa, synthetic construct
GTVTPTPNTG

SEQ ID NO: 142 - protein, 9 aa, synthetic construct
GTVTPTPNT

SEQ ID NO: 143 - protein, 8 aa, synthetic construct
GTVTPTPN

SEQ ID NO: 144 - protein, 7 aa, synthetic construct
GTVTPTP

SEQ ID NO: 145 - protein, 6 aa, synthetic construct
GTVTPT

SEQ ID NO: 146 - protein, 5 aa, synthetic construct
GTVTP

SEQ ID NO: 147 - protein, 9 aa, synthetic construct
TVTPTPNTG

SEQ ID NO: 148 - protein, 8 aa, synthetic construct
TVTPTPNT

SEQ ID NO: 149 - protein, 7 aa, synthetic construct
TVTPTPN

SEQ ID NO: 150 - protein, 6 aa, synthetic construct
TVTPTP

SEQ ID NO: 151 - protein, 5 aa, synthetic construct
TVTPT

SEQ ID NO: 152 - protein, 8 aa, synthetic construct
VTPTPNTG

SEQ ID NO: 153 - protein, 7 aa, synthetic construct
VTPTPNT

SEQ ID NO: 154 - protein, 6 aa, synthetic construct
VTPTPN

SEQ ID NO: 155 - protein, 5 aa, synthetic construct
VTPTP

SEQ ID NO: 156 - protein, 7 aa, synthetic construct
TPTPNTG

SEQ ID NO: 157 - protein, 6 aa, synthetic construct
TPTPNT

SEQ ID NO: 158 - protein, 5 aa, synthetic construct
TPTPN

SEQ ID NO: 159 - protein, 6 aa, synthetic construct
PTPNTG

SEQ ID NO: 160 - protein, 5 aa, synthetic construct
PTPNT

SEQ ID NO: 161 - protein, 5 aa, synthetic construct
TPNTG